European Patent Application EP 4 570 911 A1, published June 18, 2025. Title: 一种表观编辑靶点的方法及用途. Applicant: 益杰立科（上海）生物科技有限公司. The sequence listing filed with the application follows.

SEQUENCE LISTING (146 sequences)

SEQ ID NO: 1 - RNA, 20 nt, synthetic construct
  modified_base 6: mod_base = OTHER; note = thymine
  modified_base 14: mod_base = OTHER; note = thymine
  modified_base 17: mod_base = OTHER; note = thymine
  misc_feature 1..20: note = mANGPTL3-1
  source 1..20: mol_type = other RNA
ggaaatgagcaactaatagg

SEQ ID NO: 2 - RNA, 20 nt, synthetic construct
  modified_base 2: mod_base = OTHER; note = thymine
  modified_base 8: mod_base = OTHER; note = thymine
  modified_base 10: mod_base = OTHER; note = thymine
  modified_base 13..14: mod_base = OTHER; note = thymine
  misc_feature 1..20: note = mANGPTL3-2
  source 1..20: mol_type = other RNA
gtccaggtctccttacagga

SEQ ID NO: 3 - RNA, 20 nt, synthetic construct
  modified_base 3: mod_base = OTHER; note = thymine
  modified_base 7: mod_base = OTHER; note = thymine
  modified_base 20: mod_base = OTHER; note = thymine
  misc_feature 1..20: note = mANGPTL3-3
  source 1..20: mol_type = other RNA
gctgcatgcacacacaaggt

SEQ ID NO: 4 - RNA, 20 nt, synthetic construct
  modified_base 2..3: mod_base = OTHER; note = thymine
  modified_base 6: mod_base = OTHER; note = thymine
  modified_base 8: mod_base = OTHER; note = thymine
  modified_base 12: mod_base = OTHER; note = thymine
  modified_base 18: mod_base = OTHER; note = thymine
  misc_feature 1..20: note = mANGPTL3-4
  source 1..20: mol_type = other RNA
attgatctaactcaacatgg

SEQ ID NO: 5 - RNA, 20 nt, synthetic construct
  modified_base 3: mod_base = OTHER; note = thymine
  modified_base 9: mod_base = OTHER; note = thymine
  modified_base 11: mod_base = OTHER; note = thymine
  modified_base 14..15: mod_base = OTHER; note = thymine
  misc_feature 1..20: note = mANGPTL3-5
  source 1..20: mol_type = other RNA
ggtccaggtctccttacagg

SEQ ID NO: 6 - RNA, 20 nt, synthetic construct
  modified_base 4..5: mod_base = OTHER; note = thymine
  modified_base 8: mod_base = OTHER; note = thymine
  modified_base 10: mod_base = OTHER; note = thymine
  modified_base 14: mod_base = OTHER; note = thymine
  modified_base 20: mod_base = OTHER; note = thymine
  misc_feature 1..20: note = mANGPTL3-6
  source 1..20: mol_type = other RNA
ccattgatctaactcaacat

SEQ ID NO: 7 - RNA, 20 nt, synthetic construct
  modified_base 5: mod_base = OTHER; note = thymine
  modified_base 7..8: mod_base = OTHER; note = thymine
  modified_base 12..13: mod_base = OTHER; note = thymine
  modified_base 17: mod_base = OTHER; note = thymine
  misc_feature 1..20: note = mANGPTL3-7
  source 1..20: mol_type = other RNA
cccatgttgagttagatcaa

SEQ ID NO: 8 - RNA, 20 nt, synthetic construct
  modified_base 1: mod_base = OTHER; note = thymine
  modified_base 8: mod_base = OTHER; note = thymine
  modified_base 10: mod_base = OTHER; note = thymine
  modified_base 14: mod_base = OTHER; note = thymine
  modified_base 19: mod_base = OTHER; note = thymine
  misc_feature 1..20: note = mANGPTL3-8
  source 1..20: mol_type = other RNA
tgaaaggtctggatccactc

SEQ ID NO: 9 - RNA, 20 nt, synthetic construct
  modified_base 1: mod_base = OTHER; note = thymine
  modified_base 5: mod_base = OTHER; note = thymine
  modified_base 9: mod_base = OTHER; note = thymine
  modified_base 18: mod_base = OTHER; note = thymine
  misc_feature 1..20: note = mANGPTL3-9
  source 1..20: mol_type = other RNA
taagtccatgacccagctgc

SEQ ID NO: 10 - RNA, 20 nt, synthetic construct
  modified_base 2: mod_base = OTHER; note = thymine
  modified_base 6: mod_base = OTHER; note = thymine
  modified_base 15: mod_base = OTHER; note = thymine
  misc_feature 1..20: note = mANGPTL3-10
  source 1..20: mol_type = other RNA
gtccatgacccagctgcagg

SEQ ID NO: 11 - RNA, 20 nt, synthetic construct
  modified_base 9..10: mod_base = OTHER; note = thymine
  misc_feature 1..20: note = mANGPTL3-11
  source 1..20: mol_type = other RNA
acacaaggttggcaggagaa

SEQ ID NO: 12 - RNA, 20 nt, synthetic construct
  modified_base 1: mod_base = OTHER; note = thymine
  modified_base 7..8: mod_base = OTHER; note = thymine
  modified_base 10: mod_base = OTHER; note = thymine
  modified_base 14: mod_base = OTHER; note = thymine
  modified_base 17: mod_base = OTHER; note = thymine
  modified_base 19: mod_base = OTHER; note = thymine
  misc_feature 1..20: note = mANGPTL3-12
  source 1..20: mol_type = other RNA
tggaacttctccctcctgta

SEQ ID NO: 13 - RNA, 20 nt, synthetic construct
  modified_base 6: mod_base = OTHER; note = thymine
  modified_base 11: mod_base = OTHER; note = thymine
  modified_base 14: mod_base = OTHER; note = thymine
  modified_base 20: mod_base = OTHER; note = thymine
  misc_feature 1..20: note = mANGPTL3-13
  source 1..20: mol_type = other RNA
gcgaatggcctcctgcagct

SEQ ID NO: 14 - RNA, 20 nt, synthetic construct
  modified_base 5: mod_base = OTHER; note = thymine
  modified_base 7: mod_base = OTHER; note = thymine
  modified_base 9: mod_base = OTHER; note = thymine
  modified_base 11: mod_base = OTHER; note = thymine
  modified_base 16: mod_base = OTHER; note = thymine
  misc_feature 1..20: note = mANGPTL3-14
  source 1..20: mol_type = other RNA
gccgtgtatataaagtcaag

SEQ ID NO: 15 - RNA, 20 nt, synthetic construct
  modified_base 2: mod_base = OTHER; note = thymine
  modified_base 9: mod_base = OTHER; note = thymine
  modified_base 14: mod_base = OTHER; note = thymine
  modified_base 17: mod_base = OTHER; note = thymine
  misc_feature 1..20: note = mANGPTL3-15
  source 1..20: mol_type = other RNA
gtgcagaatcaaatgatgaa

SEQ ID NO: 16 - RNA, 20 nt, synthetic construct
  modified_base 4: mod_base = OTHER; note = thymine
  modified_base 9: mod_base = OTHER; note = thymine
  modified_base 12: mod_base = OTHER; note = thymine
  modified_base 19: mod_base = OTHER; note = thymine
  misc_feature 1..20: note = mANGPTL3-16
  source 1..20: mol_type = other RNA
gaatcaaatgatgaaaggtc

SEQ ID NO: 17 - RNA, 20 nt, synthetic construct
  modified_base 3..4: mod_base = OTHER; note = thymine
  modified_base 7: mod_base = OTHER; note = thymine
  modified_base 9: mod_base = OTHER; note = thymine
  modified_base 13: mod_base = OTHER; note = thymine
  modified_base 19: mod_base = OTHER; note = thymine
  misc_feature 1..20: note = mANGPTL3-17
  source 1..20: mol_type = other RNA
cattgatctaactcaacatg

SEQ ID NO: 18 - RNA, 20 nt, synthetic construct
  modified_base 5: mod_base = OTHER; note = thymine
  modified_base 8: mod_base = OTHER; note = thymine
  modified_base 14: mod_base = OTHER; note = thymine
  modified_base 18: mod_base = OTHER; note = thymine
  misc_feature 1..20: note = mANGPTL3-18
  source 1..20: mol_type = other RNA
ggcctcctgcagctgggtca

SEQ ID NO: 19 - RNA, 20 nt, synthetic construct
  modified_base 2..4: mod_base = OTHER; note = thymine
  modified_base 7: mod_base = OTHER; note = thymine
  modified_base 11: mod_base = OTHER; note = thymine
  misc_feature 1..20: note = mANGPTL3-19
  source 1..20: mol_type = other RNA
atttgctgcatgcacacaca

SEQ ID NO: 20 - RNA, 20 nt, synthetic construct
  modified_base 5..6: mod_base = OTHER; note = thymine
  modified_base 9: mod_base = OTHER; note = thymine
  modified_base 11: mod_base = OTHER; note = thymine
  modified_base 15: mod_base = OTHER; note = thymine
  misc_feature 1..20: note = mANGPTL3-20
  source 1..20: mol_type = other RNA
gccattgatctaactcaaca

SEQ ID NO: 21 - RNA, 20 nt, synthetic construct
  modified_base 5..6: mod_base = OTHER; note = thymine
  modified_base 9: mod_base = OTHER; note = thymine
  modified_base 11: mod_base = OTHER; note = thymine
  modified_base 15: mod_base = OTHER; note = thymine
  modified_base 19: mod_base = OTHER; note = thymine
  misc_feature 1..20: note = hANGPTL3-1
  source 1..20: mol_type = other RNA
agcattgatctaactcaatg

SEQ ID NO: 22 - RNA, 20 nt, synthetic construct
  modified_base 9: mod_base = OTHER; note = thymine
  modified_base 19: mod_base = OTHER; note = thymine
  misc_feature 1..20: note = hANGPTL3-2
  source 1..20: mol_type = other RNA
gagagccgtaacaccacctg

SEQ ID NO: 23 - RNA, 20 nt, synthetic construct
  modified_base 8: mod_base = OTHER; note = thymine
  modified_base 18: mod_base = OTHER; note = thymine
  misc_feature 1..20: note = hANGPTL3-3
  source 1..20: mol_type = other RNA
agagccgtaacaccacctga

SEQ ID NO: 24 - RNA, 20 nt, synthetic construct
  modified_base 3..5: mod_base = OTHER; note = thymine
  modified_base 7..8: mod_base = OTHER; note = thymine
  modified_base 10..11: mod_base = OTHER; note = thymine
  modified_base 16..17: mod_base = OTHER; note = thymine
  misc_feature 1..20: note = hANGPTL3-4
  source 1..20: mol_type = other RNA
aatttattattaaagttgag

SEQ ID NO: 25 - RNA, 20 nt, synthetic construct
  modified_base 3: mod_base = OTHER; note = thymine
  modified_base 9: mod_base = OTHER; note = thymine
  modified_base 16: mod_base = OTHER; note = thymine
  misc_feature 1..20: note = hANGPTL3-5
  source 1..20: mol_type = other RNA
actacaagtcaaaaatgaag

SEQ ID NO: 26 - RNA, 20 nt, synthetic construct
  modified_base 5: mod_base = OTHER; note = thymine
  modified_base 11..12: mod_base = OTHER; note = thymine
  modified_base 16: mod_base = OTHER; note = thymine
  modified_base 19: mod_base = OTHER; note = thymine
  misc_feature 1..20: note = hANGPTL3-6
  source 1..20: mol_type = other RNA
aaactacacattcaatgcta

SEQ ID NO: 27 - RNA, 20 nt, synthetic construct
  modified_base 2: mod_base = OTHER; note = thymine
  modified_base 7..12: mod_base = OTHER; note = thymine
  modified_base 14..15: mod_base = OTHER; note = thymine
  modified_base 17: mod_base = OTHER; note = thymine
  misc_feature 1..20: note = hANGPTL3-7
  source 1..20: mol_type = other RNA
gtagaattttttcttctagg

SEQ ID NO: 28 - RNA, 20 nt, synthetic construct
  modified_base 11: mod_base = OTHER; note = thymine
  modified_base 16..17: mod_base = OTHER; note = thymine
  modified_base 20: mod_base = OTHER; note = thymine
  misc_feature 1..20: note = hANGPTL3-8
  source 1..20: mol_type = other RNA
ccagaaaaggtaaggttggt

SEQ ID NO: 29 - RNA, 20 nt, synthetic construct
  modified_base 1: mod_base = OTHER; note = thymine
  modified_base 5..6: mod_base = OTHER; note = thymine
  modified_base 9: mod_base = OTHER; note = thymine
  modified_base 15..16: mod_base = OTHER; note = thymine
  misc_feature 1..20: note = hANGPTL3-9
  source 1..20: mol_type = other RNA
tacattcgtgcaagttaaca

SEQ ID NO: 30 - RNA, 20 nt, synthetic construct
  modified_base 3: mod_base = OTHER; note = thymine
  modified_base 13: mod_base = OTHER; note = thymine
  misc_feature 1..20: note = hANGPTL3-10
  source 1..20: mol_type = other RNA
cgtaacaccacctgagggag

SEQ ID NO: 31 - RNA, 20 nt, synthetic construct
  modified_base 2: mod_base = OTHER; note = thymine
  modified_base 4: mod_base = OTHER; note = thymine
  modified_base 8: mod_base = OTHER; note = thymine
  modified_base 12: mod_base = OTHER; note = thymine
  modified_base 14: mod_base = OTHER; note = thymine
  misc_feature 1..20: note = hANGPTL3-11
  source 1..20: mol_type = other RNA
atctaactcaatgtggaaga

SEQ ID NO: 32 - RNA, 20 nt, synthetic construct
  modified_base 1: mod_base = OTHER; note = thymine
  modified_base 5..7: mod_base = OTHER; note = thymine
  modified_base 9..10: mod_base = OTHER; note = thymine
  modified_base 12..13: mod_base = OTHER; note = thymine
  modified_base 18..19: mod_base = OTHER; note = thymine
  misc_feature 1..20: note = hANGPTL3-12
  source 1..20: mol_type = other RNA
taaatttattattaaagttg

SEQ ID NO: 33 - RNA, 20 nt, synthetic construct
  modified_base 3..5: mod_base = OTHER; note = thymine
  modified_base 7: mod_base = OTHER; note = thymine
  modified_base 12: mod_base = OTHER; note = thymine
  modified_base 16: mod_base = OTHER; note = thymine
  misc_feature 1..20: note = hANGPTL3-13
  source 1..20: mol_type = other RNA
cctttctccactccctcagg

SEQ ID NO: 34 - RNA, 20 nt, synthetic construct
  modified_base 2..3: mod_base = OTHER; note = thymine
  modified_base 5: mod_base = OTHER; note = thymine
  modified_base 7..8: mod_base = OTHER; note = thymine
  modified_base 11: mod_base = OTHER; note = thymine
  modified_base 15..16: mod_base = OTHER; note = thymine
  modified_base 18: mod_base = OTHER; note = thymine
  misc_feature 1..20: note = hANGPTL3-14
  source 1..20: mol_type = other RNA
attgtcttgatcaattctgg

SEQ ID NO: 35 - RNA, 20 nt, synthetic construct
  modified_base 4: mod_base = OTHER; note = thymine
  modified_base 8: mod_base = OTHER; note = thymine
  modified_base 13: mod_base = OTHER; note = thymine
  modified_base 16: mod_base = OTHER; note = thymine
  modified_base 18..19: mod_base = OTHER; note = thymine
  misc_feature 1..20: note = hANGPTL3-15
  source 1..20: mol_type = other RNA
cactccctcaggtggtgtta

SEQ ID NO: 36 - RNA, 20 nt, synthetic construct
  modified_base 4..6: mod_base = OTHER; note = thymine
  modified_base 8: mod_base = OTHER; note = thymine
  modified_base 12: mod_base = OTHER; note = thymine
  misc_feature 1..20: note = hANGPTL3-16
  source 1..20: mol_type = other RNA
gactttgtccataagacgaa

SEQ ID NO: 37 - RNA, 20 nt, synthetic construct
  modified_base 2: mod_base = OTHER; note = thymine
  modified_base 4: mod_base = OTHER; note = thymine
  modified_base 8: mod_base = OTHER; note = thymine
  modified_base 11: mod_base = OTHER; note = thymine
  modified_base 13: mod_base = OTHER; note = thymine
  modified_base 15..16: mod_base = OTHER; note = thymine
  modified_base 19: mod_base = OTHER; note = thymine
  misc_feature 1..20: note = hANGPTL3-17
  source 1..20: mol_type = other RNA
ctctcaatgctgtgttcctc

SEQ ID NO: 38 - RNA, 20 nt, synthetic construct
  modified_base 2..5: mod_base = OTHER; note = thymine
  modified_base 9..11: mod_base = OTHER; note = thymine
  misc_feature 1..20: note = hANGPTL3-18
  source 1..20: mol_type = other RNA
attttcaatttcaagcaacg

SEQ ID NO: 39 - RNA, 20 nt, synthetic construct
  modified_base 4: mod_base = OTHER; note = thymine
  modified_base 12: mod_base = OTHER; note = thymine
  modified_base 16..17: mod_base = OTHER; note = thymine
  modified_base 20: mod_base = OTHER; note = thymine
  misc_feature 1..20: note = hANGPTL3-19
  source 1..20: mol_type = other RNA
aaatgagcaactaacttaat

SEQ ID NO: 40 - RNA, 20 nt, synthetic construct
  modified_base 6: mod_base = OTHER; note = thymine
  modified_base 14: mod_base = OTHER; note = thymine
  misc_feature 1..20: note = hANGPTL3-20
  source 1..20: mol_type = other RNA
ccacctgagggagtggagaa

SEQ ID NO: 41 - RNA, 20 nt, synthetic construct
  modified_base 5..7: mod_base = OTHER; note = thymine
  modified_base 9: mod_base = OTHER; note = thymine
  modified_base 13: mod_base = OTHER; note = thymine
  misc_feature 1..20: note = hANGPTL3-21
  source 1..20: mol_type = other RNA
agactttgtccataagacga

SEQ ID NO: 42 - RNA, 20 nt, synthetic construct
  modified_base 1..2: mod_base = OTHER; note = thymine
  modified_base 15: mod_base = OTHER; note = thymine
  modified_base 20: mod_base = OTHER; note = thymine
  misc_feature 1..20: note = hANGPTL3-22
  source 1..20: mol_type = other RNA
ttgcccagaaaaggtaaggt

SEQ ID NO: 43 - RNA, 20 nt, synthetic construct
  modified_base 1: mod_base = OTHER; note = thymine
  modified_base 8: mod_base = OTHER; note = thymine
  modified_base 20: mod_base = OTHER; note = thymine
  misc_feature 1..20: note = hANGPTL3-23
  source 1..20: mol_type = other RNA
tcccaactgaaggaggccat

SEQ ID NO: 44 - RNA, 20 nt, synthetic construct
  modified_base 6..8: mod_base = OTHER; note = thymine
  modified_base 10: mod_base = OTHER; note = thymine
  modified_base 15: mod_base = OTHER; note = thymine
  modified_base 19: mod_base = OTHER; note = thymine
  misc_feature 1..20: note = hANGPTL3-24
  source 1..20: mol_type = other RNA
aagcctttctccactccctc

SEQ ID NO: 45 - RNA, 20 nt, synthetic construct
  modified_base 1..2: mod_base = OTHER; note = thymine
  modified_base 4..5: mod_base = OTHER; note = thymine
  modified_base 7..8: mod_base = OTHER; note = thymine
  modified_base 10..12: mod_base = OTHER; note = thymine
  modified_base 15..17: mod_base = OTHER; note = thymine
  misc_feature 1..20: note = hANGPTL3-25
  source 1..20: mol_type = other RNA
ttcttcttctttgatttcac

SEQ ID NO: 46 - RNA, 20 nt, synthetic construct
  modified_base 9: mod_base = OTHER; note = thymine
  modified_base 11..16: mod_base = OTHER; note = thymine
  misc_feature 1..20: note = hANGPTL3-26
  source 1..20: mol_type = other RNA
agagaaagtgttttttggaa

SEQ ID NO: 47 - RNA, 20 nt, synthetic construct
  modified_base 1: mod_base = OTHER; note = thymine
  modified_base 6..7: mod_base = OTHER; note = thymine
  modified_base 11..14: mod_base = OTHER; note = thymine
  misc_feature 1..20: note = hANGPTL3-27
  source 1..20: mol_type = other RNA
taaaattagcttttaaaaac

SEQ ID NO: 48 - RNA, 20 nt, synthetic construct
  modified_base 4..6: mod_base = OTHER; note = thymine
  modified_base 8..9: mod_base = OTHER; note = thymine
  modified_base 11..12: mod_base = OTHER; note = thymine
  modified_base 17..18: mod_base = OTHER; note = thymine
  misc_feature 1..20: note = hANGPTL3-28
  source 1..20: mol_type = other RNA
aaatttattattaaagttga

SEQ ID NO: 49 - RNA, 20 nt, synthetic construct
  modified_base 2..3: mod_base = OTHER; note = thymine
  modified_base 5: mod_base = OTHER; note = thymine
  modified_base 14: mod_base = OTHER; note = thymine
  modified_base 18: mod_base = OTHER; note = thymine
  misc_feature 1..20: note = hANGPTL3-29
  source 1..20: mol_type = other RNA
attctggaggaaataactag

SEQ ID NO: 50 - RNA, 20 nt, synthetic construct
  modified_base 1: mod_base = OTHER; note = thymine
  modified_base 9: mod_base = OTHER; note = thymine
  modified_base 11: mod_base = OTHER; note = thymine
  modified_base 18: mod_base = OTHER; note = thymine
  misc_feature 1..20: note = hANGPTL3-30
  source 1..20: mol_type = other RNA
taagaccatgtcccaactga

SEQ ID NO: 51 - RNA, 20 nt, synthetic construct
  modified_base 1: mod_base = OTHER; note = thymine
  modified_base 6: mod_base = OTHER; note = thymine
  misc_feature 1..20: note = hANGPTL3-31
  source 1..20: mol_type = other RNA
tgaaatcaaagaagaagaaa

SEQ ID NO: 52 - RNA, 20 nt, synthetic construct
  modified_base 3: mod_base = OTHER; note = thymine
  modified_base 5: mod_base = OTHER; note = thymine
  modified_base 11..14: mod_base = OTHER; note = thymine
  misc_feature 1..20: note = hANGPTL3-32
  source 1..20: mol_type = other RNA
gatgtaaaaattttagccaa

SEQ ID NO: 53 - RNA, 20 nt, synthetic construct
  modified_base 5: mod_base = OTHER; note = thymine
  modified_base 7: mod_base = OTHER; note = thymine
  modified_base 10..12: mod_base = OTHER; note = thymine
  modified_base 15..16: mod_base = OTHER; note = thymine
  modified_base 18..20: mod_base = OTHER; note = thymine
  misc_feature 1..20: note = hANGPTL3-33
  source 1..20: mol_type = other RNA
aaactgtactttagttcttt

SEQ ID NO: 54 - RNA, 20 nt, synthetic construct
  modified_base 2: mod_base = OTHER; note = thymine
  modified_base 4..6: mod_base = OTHER; note = thymine
  modified_base 19: mod_base = OTHER; note = thymine
  misc_feature 1..20: note = hANGPTL3-34
  source 1..20: mol_type = other RNA
atatttgcccagaaaaggta

SEQ ID NO: 55 - RNA, 20 nt, synthetic construct
  modified_base 6: mod_base = OTHER; note = thymine
  modified_base 8: mod_base = OTHER; note = thymine
  modified_base 15: mod_base = OTHER; note = thymine
  misc_feature 1..20: note = hANGPTL3-35
  source 1..20: mol_type = other RNA
gaccatgtcccaactgaagg

SEQ ID NO: 56 - RNA, 20 nt, synthetic construct
  modified_base 5: mod_base = OTHER; note = thymine
  modified_base 8..9: mod_base = OTHER; note = thymine
  modified_base 13..14: mod_base = OTHER; note = thymine
  misc_feature 1..20: note = hANGPTL3-36
  source 1..20: mol_type = other RNA
ggcctccttcagttgggaca

SEQ ID NO: 57 - RNA, 20 nt, synthetic construct
  modified_base 7: mod_base = OTHER; note = thymine
  modified_base 12: mod_base = OTHER; note = thymine
  modified_base 15..16: mod_base = OTHER; note = thymine
  modified_base 20: mod_base = OTHER; note = thymine
  misc_feature 1..20: note = hANGPTL3-37
  source 1..20: mol_type = other RNA
agccaatggcctccttcagt

SEQ ID NO: 58 - RNA, 20 nt, synthetic construct
  modified_base 1: mod_base = OTHER; note = thymine
  modified_base 5..6: mod_base = OTHER; note = thymine
  modified_base 8: mod_base = OTHER; note = thymine
  modified_base 10..11: mod_base = OTHER; note = thymine
  modified_base 14: mod_base = OTHER; note = thymine
  modified_base 18..19: mod_base = OTHER; note = thymine
  misc_feature 1..20: note = hANGPTL3-38
  source 1..20: mol_type = other RNA
tgaattgtcttgatcaattc

SEQ ID NO: 59 - RNA, 20 nt, synthetic construct
  modified_base 2: mod_base = OTHER; note = thymine
  modified_base 13: mod_base = OTHER; note = thymine
  misc_feature 1..20: note = hANGPTL3-39
  source 1..20: mol_type = other RNA
ctagaggaacaataaaaaga

SEQ ID NO: 60 - RNA, 20 nt, synthetic construct
  modified_base 1: mod_base = OTHER; note = thymine
  modified_base 3: mod_base = OTHER; note = thymine
  modified_base 5: mod_base = OTHER; note = thymine
  modified_base 10..11: mod_base = OTHER; note = thymine
  modified_base 18: mod_base = OTHER; note = thymine
  modified_base 20: mod_base = OTHER; note = thymine
  misc_feature 1..20: note = hANGPTL3-40
  source 1..20: mol_type = other RNA
tatatagagttaagaagtct

SEQ ID NO: 61 - RNA, 20 nt, synthetic construct
  modified_base 1: mod_base = OTHER; note = thymine
  modified_base 4..6: mod_base = OTHER; note = thymine
  modified_base 12..13: mod_base = OTHER; note = thymine
  modified_base 16: mod_base = OTHER; note = thymine
  modified_base 18..19: mod_base = OTHER; note = thymine
  misc_feature 1..20: note = hANGPTL3-41
  source 1..20: mol_type = other RNA
taatttggcccttcgtctta

SEQ ID NO: 62 - RNA, 20 nt, synthetic construct
  modified_base 1: mod_base = OTHER; note = thymine
  modified_base 7: mod_base = OTHER; note = thymine
  modified_base 9..11: mod_base = OTHER; note = thymine
  misc_feature 1..20: note = hANGPTL3-42
  source 1..20: mol_type = other RNA
taccaatatttgcccagaaa

SEQ ID NO: 63 - RNA, 20 nt, synthetic construct
  modified_base 6: mod_base = OTHER; note = thymine
  modified_base 11: mod_base = OTHER; note = thymine
  modified_base 14..15: mod_base = OTHER; note = thymine
  modified_base 19..20: mod_base = OTHER; note = thymine
  misc_feature 1..20: note = hANGPTL3-43
  source 1..20: mol_type = other RNA
gccaatggcctccttcagtt

SEQ ID NO: 64 - RNA, 20 nt, synthetic construct
  modified_base 6: mod_base = OTHER; note = thymine
  modified_base 8..9: mod_base = OTHER; note = thymine
  modified_base 12..15: mod_base = OTHER; note = thymine
  modified_base 19: mod_base = OTHER; note = thymine
  misc_feature 1..20: note = hANGPTL3-44
  source 1..20: mol_type = other RNA
gcaaatcttgattttggctc

SEQ ID NO: 65 - RNA, 20 nt, synthetic construct
  modified_base 1: mod_base = OTHER; note = thymine
  modified_base 5..8: mod_base = OTHER; note = thymine
  modified_base 10: mod_base = OTHER; note = thymine
  modified_base 18: mod_base = OTHER; note = thymine
  modified_base 20: mod_base = OTHER; note = thymine
  misc_feature 1..20: note = hANGPTL3-45
  source 1..20: mol_type = other RNA
taccttttctgggcaaatat

SEQ ID NO: 66 - RNA, 20 nt, synthetic construct
  modified_base 3: mod_base = OTHER; note = thymine
  modified_base 11..12: mod_base = OTHER; note = thymine
  modified_base 16..19: mod_base = OTHER; note = thymine
  misc_feature 1..20: note = hANGPTL3-46
  source 1..20: mol_type = other RNA
cctaccaaccttaccttttc

SEQ ID NO: 67 - RNA, 20 nt, synthetic construct
  modified_base 5: mod_base = OTHER; note = thymine
  modified_base 11: mod_base = OTHER; note = thymine
  modified_base 13..16: mod_base = OTHER; note = thymine
  modified_base 18..19: mod_base = OTHER; note = thymine
  misc_feature 1..20: note = hANGPTL3-47
  source 1..20: mol_type = other RNA
aacgtggaactgttttcttc

SEQ ID NO: 68 - RNA, 20 nt, synthetic construct
  modified_base 1..3: mod_base = OTHER; note = thymine
  modified_base 8: mod_base = OTHER; note = thymine
  modified_base 10: mod_base = OTHER; note = thymine
  modified_base 12: mod_base = OTHER; note = thymine
  modified_base 15..16: mod_base = OTHER; note = thymine
  modified_base 19..20: mod_base = OTHER; note = thymine
  misc_feature 1..20: note = hANGPTL3-48
  source 1..20: mol_type = other RNA
tttgaaatatgtcattaatt

SEQ ID NO: 69 - RNA, 20 nt, synthetic construct
  modified_base 2: mod_base = OTHER; note = thymine
  modified_base 10..11: mod_base = OTHER; note = thymine
  modified_base 15..18: mod_base = OTHER; note = thymine
  modified_base 20: mod_base = OTHER; note = thymine
  misc_feature 1..20: note = hANGPTL3-49
  source 1..20: mol_type = other RNA
ctaccaaccttaccttttct

SEQ ID NO: 70 - RNA, 20 nt, synthetic construct
  modified_base 5: mod_base = OTHER; note = thymine
  modified_base 12: mod_base = OTHER; note = thymine
  modified_base 14..15: mod_base = OTHER; note = thymine
  modified_base 18..20: mod_base = OTHER; note = thymine
  misc_feature 1..20: note = hANGPTL3-50
  source 1..20: mol_type = other RNA
aacatagcaaatcttgattt

SEQ ID NO: 71 - DNA, 1000 bp, synthetic construct
  misc_feature 1..1000: note = mANGPTL3 subregion
  source 1..1000: mol_type = other DNA
ttatccgacgacagaaacagaggctatagcattgagagccgcagcactaactcaacaacttggaaagacttggggagtggttgctgtttccagataaacaaactacaaacagggttacagatgcttaatttttcctcaagctaaggaaactcacacttaagtttaatgacaaacttaatccatcaaaaactaaggtttatttgtaaatctcttatagtaagaaaaaatttaaatgatcttttaaaaacaggtaaatacctttatcctgaaagaataattatcaatacagcaaatttaactattttaacaattttgaaaattacctcctattagttgctcatttccttgatttcagttgccattgatctaactcaacatgggggagggttacattcgtgcaagttagcacagcttaatggttaactccattctcctgccaaccttgtgtgtgcatgcagcaaatagccgtgtatataaagtcaagaggtccaggtctccttacaggagggagaagttccaaattgcttaaaattgaataattgagacaaaaaatgcacacaattaaattattcctttttgttgttcctttagtaattgcatccagagtggatccagacctttcatcatttgattctgcaccttcagagccaaaatcaagatttgctatgttggatgatgtcaaaattttagcgaatggcctcctgcagctgggtcatggacttaaagattttgtccataagactaagggacaaattaacgacatatttcagaagctcaacatatttgatcagtctttttatgacctatcacttcgaaccaatgaaatcaaagaagaggaaaaggagctaagaagaactacatctacactacaagttaaaaacgaggaggtgaagaacatgtcagtagaactgaactcaaagcttgagagtctgctggaagagaagacagcccttcaacacaaggtcagggctttggaggagcagctaaccaacttaattct

SEQ ID NO: 72 - DNA, 1000 bp, synthetic construct
  misc_feature 1..1000: note = hANGPTL3 subregion
  source 1..1000: mol_type = other DNA
tacagagtaccagaggaacacagcattgagagccgtaacaccacctgagggagtggagaaaggcttcagagagaaagtgttttttggaatggatcactgtttccaaaagaactaaagtacagtttgagaaatgcatacttaattcattacttttttcccctcaactttaataataaatttacccaacaaaaaagtttatttttgacttgtaaatctcttaaaatcataaaaaagtaaaattagcttttaaaaacaggtagtcaccatagcattgaatgtgtagtttataatacagcaaagttaaatacaatttcaaattacctattaagttagttgctcatttctttgatttcatttagcattgatctaactcaatgtggaagaaggttacattcgtgcaagttaacacggcttaatgattaactatgttcacctaccaaccttaccttttctgggcaaatattggtatatatagagttaagaagtctaggtctgcttccagaagaaaacagttccacgttgcttgaaattgaaaatcaagataaaaatgttcacaattaagctccttctttttattgttcctctagttatttcctccagaattgatcaagacaattcatcatttgattctctatctccagagccaaaatcaagatttgctatgttagacgatgtaaaaattttagccaatggcctccttcagttgggacatggtcttaaagactttgtccataagacgaagggccaaattaatgacatatttcaaaaactcaacatatttgatcagtctttttatgatctatcgctgcaaaccagtgaaatcaaagaagaagaaaaggaactgagaagaactacatataaactacaagtcaaaaatgaagaggtaaagaatatgtcacttgaactcaactcaaaacttgaaagcctcctagaagaaaaaattctacttcaacaaaaagtgaaatatttagaagagcaactaactaacttaattcaaaat

SEQ ID NO: 73 - DNA, 80 bp, synthetic construct
  misc_feature 1..80: note = mANGPTL3-1 target
  source 1..80: mol_type = other DNA
ttgagttagatcaatggcaactgaaatcaaggaaatgagcaactaataggaggtaattttcaaaattgttaaaatagtta

SEQ ID NO: 74 - DNA, 80 bp, synthetic construct
  misc_feature 1..80: note = mANGPTL3-2 target
  source 1..80: mol_type = other DNA
agcaaatagccgtgtatataaagtcaagaggtccaggtctccttacaggagggagaagttccaaattgcttaaaattgaa

SEQ ID NO: 75 - DNA, 80 bp, synthetic construct
  misc_feature 1..80: note = mANGPTL3-3 target
  source 1..80: mol_type = other DNA
gacctcttgactttatatacacggctatttgctgcatgcacacacaaggttggcaggagaatggagttaaccattaagct

SEQ ID NO: 76 - DNA, 80 bp, synthetic construct
  misc_feature 1..80: note = mANGPTL3-4 target
  source 1..80: mol_type = other DNA
tagttgctcatttccttgatttcagttgccattgatctaactcaacatgggggagggttacattcgtgcaagttagcaca

SEQ ID NO: 77 - DNA, 80 bp, synthetic construct
  misc_feature 1..80: note = mANGPTL3-5 target
  source 1..80: mol_type = other DNA
cagcaaatagccgtgtatataaagtcaagaggtccaggtctccttacaggagggagaagttccaaattgcttaaaattga

SEQ ID NO: 78 - DNA, 80 bp, synthetic construct
  misc_feature 1..80: note = mANGPTL3-6 target
  source 1..80: mol_type = other DNA
attagttgctcatttccttgatttcagttgccattgatctaactcaacatgggggagggttacattcgtgcaagttagca

SEQ ID NO: 79 - DNA, 80 bp, synthetic construct
  misc_feature 1..80: note = mANGPTL3-7 target
  source 1..80: mol_type = other DNA
ctgtgctaacttgcacgaatgtaaccctcccccatgttgagttagatcaatggcaactgaaatcaaggaaatgagcaact

SEQ ID NO: 80 - DNA, 80 bp, synthetic construct
  misc_feature 1..80: note = mANGPTL3-8 target
  source 1..80: mol_type = other DNA
ttttggctctgaaggtgcagaatcaaatgatgaaaggtctggatccactctggatgcaattactaaaggaacaacaaaaa

SEQ ID NO: 81 - DNA, 80 bp, synthetic construct
  misc_feature 1..80: note = mANGPTL3-9 target
  source 1..80: mol_type = other DNA
tttgtcccttagtcttatggacaaaatctttaagtccatgacccagctgcaggaggccattcgctaaaattttgacatca

SEQ ID NO: 82 - DNA, 80 bp, synthetic construct
  misc_feature 1..80: note = mANGPTL3-10 target
  source 1..80: mol_type = other DNA
gtcccttagtcttatggacaaaatctttaagtccatgacccagctgcaggaggccattcgctaaaattttgacatcatcc

SEQ ID NO: 83 - DNA, 80 bp, synthetic construct
  misc_feature 1..80: note = mANGPTL3-11 target
  source 1..80: mol_type = other DNA
tttatatacacggctatttgctgcatgcacacacaaggttggcaggagaatggagttaaccattaagctgtgctaacttg

SEQ ID NO: 84 - DNA, 80 bp, synthetic construct
  misc_feature 1..80: note = mANGPTL3-12 target
  source 1..80: mol_type = other DNA
tttgtctcaattattcaattttaagcaatttggaacttctccctcctgtaaggagacctggacctcttgactttatatac

SEQ ID NO: 85 - DNA, 80 bp, synthetic construct
  misc_feature 1..80: note = mANGPTL3-13 target
  source 1..80: mol_type = other DNA
tttgctatgttggatgatgtcaaaattttagcgaatggcctcctgcagctgggtcatggacttaaagattttgtccataa

SEQ ID NO: 86 - DNA, 80 bp, synthetic construct
  misc_feature 1..80: note = mANGPTL3-14 target
  source 1..80: mol_type = other DNA
tgccaaccttgtgtgtgcatgcagcaaatagccgtgtatataaagtcaagaggtccaggtctccttacaggagggagaag

SEQ ID NO: 87 - DNA, 80 bp, synthetic construct
  misc_feature 1..80: note = mANGPTL3-15 target
  source 1..80: mol_type = other DNA
acatagcaaatcttgattttggctctgaaggtgcagaatcaaatgatgaaaggtctggatccactctggatgcaattact

SEQ ID NO: 88 - DNA, 80 bp, synthetic construct
  misc_feature 1..80: note = mANGPTL3-16 target
  source 1..80: mol_type = other DNA
gcaaatcttgattttggctctgaaggtgcagaatcaaatgatgaaaggtctggatccactctggatgcaattactaaagg

SEQ ID NO: 89 - DNA, 80 bp, synthetic construct
  misc_feature 1..80: note = mANGPTL3-17 target
  source 1..80: mol_type = other DNA
ttagttgctcatttccttgatttcagttgccattgatctaactcaacatgggggagggttacattcgtgcaagttagcac

SEQ ID NO: 90 - DNA, 80 bp, synthetic construct
  misc_feature 1..80: note = mANGPTL3-18 target
  source 1..80: mol_type = other DNA
atgttggatgatgtcaaaattttagcgaatggcctcctgcagctgggtcatggacttaaagattttgtccataagactaa

SEQ ID NO: 91 - DNA, 80 bp, synthetic construct
  misc_feature 1..80: note = mANGPTL3-19 target
  source 1..80: mol_type = other DNA
cctggacctcttgactttatatacacggctatttgctgcatgcacacacaaggttggcaggagaatggagttaaccatta

SEQ ID NO: 92 - DNA, 80 bp, synthetic construct
  misc_feature 1..80: note = mANGPTL3-20 target
  source 1..80: mol_type = other DNA
tattagttgctcatttccttgatttcagttgccattgatctaactcaacatgggggagggttacattcgtgcaagttagc

SEQ ID NO: 93 - DNA, 80 bp, synthetic construct
  misc_feature 1..80: note = hANGPTL3-1 target
  source 1..80: mol_type = other DNA
agttagttgctcatttctttgatttcatttagcattgatctaactcaatgtggaagaaggttacattcgtgcaagttaac

SEQ ID NO: 94 - DNA, 78 bp, synthetic construct
  misc_feature 1..78: note = hANGPTL3-2 target
  source 1..78: mol_type = other DNA
tacagagtaccagaggaacacagcattgagagccgtaacaccacctgagggagtggagaaaggcttcagagagaaagt

SEQ ID NO: 95 - DNA, 79 bp, synthetic construct
  misc_feature 1..79: note = hANGPTL3-3 target
  source 1..79: mol_type = other DNA
tacagagtaccagaggaacacagcattgagagccgtaacaccacctgagggagtggagaaaggcttcagagagaaagtg

SEQ ID NO: 96 - DNA, 80 bp, synthetic construct
  misc_feature 1..80: note = hANGPTL3-4 target
  source 1..80: mol_type = other DNA
caagtcaaaaataaacttttttgttgggtaaatttattattaaagttgaggggaaaaaagtaatgaattaagtatgcatt

SEQ ID NO: 97 - DNA, 80 bp, synthetic construct
  misc_feature 1..80: note = hANGPTL3-5 target
  source 1..80: mol_type = other DNA
agaaaaggaactgagaagaactacatataaactacaagtcaaaaatgaagaggtaaagaatatgtcacttgaactcaact

SEQ ID NO: 98 - DNA, 80 bp, synthetic construct
  misc_feature 1..80: note = hANGPTL3-6 target
  source 1..80: mol_type = other DNA
ttgaaattgtatttaactttgctgtattataaactacacattcaatgctatggtgactacctgtttttaaaagctaattt

SEQ ID NO: 99 - DNA, 80 bp, synthetic construct
  misc_feature 1..80: note = hANGPTL3-7 target
  source 1..80: mol_type = other DNA
gctcttctaaatatttcactttttgttgaagtagaattttttcttctaggaggctttcaagttttgagttgagttcaagt

SEQ ID NO: 100 - DNA, 80 bp, synthetic construct
  misc_feature 1..80: note = hANGPTL3-8 target
  source 1..80: mol_type = other DNA
cttcttaactctatatataccaatatttgcccagaaaaggtaaggttggtaggtgaacatagttaatcattaagccgtgt

SEQ ID NO: 101 - DNA, 80 bp, synthetic construct
  misc_feature 1..80: note = hANGPTL3-9 target
  source 1..80: mol_type = other DNA
gcattgatctaactcaatgtggaagaaggttacattcgtgcaagttaacacggcttaatgattaactatgttcacctacc

SEQ ID NO: 102 - DNA, 80 bp, synthetic construct
  misc_feature 1..80: note = hANGPTL3-10 target
  source 1..80: mol_type = other DNA
agagtaccagaggaacacagcattgagagccgtaacaccacctgagggagtggagaaaggcttcagagagaaagtgtttt

SEQ ID NO: 103 - DNA, 80 bp, synthetic construct
  misc_feature 1..80: note = hANGPTL3-11 target
  source 1..80: mol_type = other DNA
tgctcatttctttgatttcatttagcattgatctaactcaatgtggaagaaggttacattcgtgcaagttaacacggctt

SEQ ID NO: 104 - DNA, 80 bp, synthetic construct
  misc_feature 1..80: note = hANGPTL3-12 target
  source 1..80: mol_type = other DNA
tacaagtcaaaaataaacttttttgttgggtaaatttattattaaagttgaggggaaaaaagtaatgaattaagtatgca

SEQ ID NO: 105 - DNA, 80 bp, synthetic construct
  misc_feature 1..80: note = hANGPTL3-13 target
  source 1..80: mol_type = other DNA
tccattccaaaaaacactttctctctgaagcctttctccactccctcaggtggtgttacggctctcaatgctgtgttcct

SEQ ID NO: 106 - DNA, 80 bp, synthetic construct
  misc_feature 1..80: note = hANGPTL3-14 target
  source 1..80: mol_type = other DNA
tggctctggagatagagaatcaaatgatgaattgtcttgatcaattctggaggaaataactagaggaacaataaaaagaa

SEQ ID NO: 107 - DNA, 80 bp, synthetic construct
  misc_feature 1..80: note = hANGPTL3-15 target
  source 1..80: mol_type = other DNA
aaaaaacactttctctctgaagcctttctccactccctcaggtggtgttacggctctcaatgctgtgttcctctggtact

SEQ ID NO: 108 - DNA, 80 bp, synthetic construct
  misc_feature 1..80: note = hANGPTL3-16 target
  source 1..80: mol_type = other DNA
ggcctccttcagttgggacatggtcttaaagactttgtccataagacgaagggccaaattaatgacatatttcaaaaact

SEQ ID NO: 109 - DNA, 62 bp, synthetic construct
  misc_feature 1..62: note = hANGPTL3-17 target
  source 1..62: mol_type = other DNA
ctttctccactccctcaggtggtgttacggctctcaatgctgtgttcctctggtactctgta

SEQ ID NO: 110 - DNA, 80 bp, synthetic construct
  misc_feature 1..80: note = hANGPTL3-18 target
  source 1..80: mol_type = other DNA
aggagcttaattgtgaacatttttatcttgattttcaatttcaagcaacgtggaactgttttcttctggaagcagaccta

SEQ ID NO: 111 - DNA, 80 bp, synthetic construct
  misc_feature 1..80: note = hANGPTL3-19 target
  source 1..80: mol_type = other DNA
gagttagatcaatgctaaatgaaatcaaagaaatgagcaactaacttaataggtaatttgaaattgtatttaactttgct

SEQ ID NO: 112 - DNA, 80 bp, synthetic construct
  misc_feature 1..80: note = hANGPTL3-20 target
  source 1..80: mol_type = other DNA
cagaggaacacagcattgagagccgtaacaccacctgagggagtggagaaaggcttcagagagaaagtgttttttggaat

SEQ ID NO: 113 - DNA, 80 bp, synthetic construct
  misc_feature 1..80: note = hANGPTL3-21 target
  source 1..80: mol_type = other DNA
tggcctccttcagttgggacatggtcttaaagactttgtccataagacgaagggccaaattaatgacatatttcaaaaac

SEQ ID NO: 114 - DNA, 80 bp, synthetic construct
  misc_feature 1..80: note = hANGPTL3-22 target
  source 1..80: mol_type = other DNA
tagacttcttaactctatatataccaatatttgcccagaaaaggtaaggttggtaggtgaacatagttaatcattaagcc

SEQ ID NO: 115 - DNA, 80 bp, synthetic construct
  misc_feature 1..80: note = hANGPTL3-23 target
  source 1..80: mol_type = other DNA
cgtcttatggacaaagtctttaagaccatgtcccaactgaaggaggccattggctaaaatttttacatcgtctaacatag

SEQ ID NO: 116 - DNA, 80 bp, synthetic construct
  misc_feature 1..80: note = hANGPTL3-24 target
  source 1..80: mol_type = other DNA
tgatccattccaaaaaacactttctctctgaagcctttctccactccctcaggtggtgttacggctctcaatgctgtgtt

SEQ ID NO: 117 - DNA, 80 bp, synthetic construct
  misc_feature 1..80: note = hANGPTL3-25 target
  source 1..80: mol_type = other DNA
tagtttatatgtagttcttctcagttccttttcttcttctttgatttcactggtttgcagcgatagatcataaaaagact

SEQ ID NO: 118 - DNA, 80 bp, synthetic construct
  misc_feature 1..80: note = hANGPTL3-26 target
  source 1..80: mol_type = other DNA
accacctgagggagtggagaaaggcttcagagagaaagtgttttttggaatggatcactgtttccaaaagaactaaagta

SEQ ID NO: 119 - DNA, 80 bp, synthetic construct
  misc_feature 1..80: note = hANGPTL3-27 target
  source 1..80: mol_type = other DNA
acttgtaaatctcttaaaatcataaaaaagtaaaattagcttttaaaaacaggtagtcaccatagcattgaatgtgtagt

SEQ ID NO: 120 - DNA, 80 bp, synthetic construct
  misc_feature 1..80: note = hANGPTL3-28 target
  source 1..80: mol_type = other DNA
acaagtcaaaaataaacttttttgttgggtaaatttattattaaagttgaggggaaaaaagtaatgaattaagtatgcat

SEQ ID NO: 121 - DNA, 80 bp, synthetic construct
  misc_feature 1..80: note = hANGPTL3-29 target
  source 1..80: mol_type = other DNA
agagaatcaaatgatgaattgtcttgatcaattctggaggaaataactagaggaacaataaaaagaaggagcttaattgt

SEQ ID NO: 122 - DNA, 80 bp, synthetic construct
  misc_feature 1..80: note = hANGPTL3-30 target
  source 1..80: mol_type = other DNA
tttggcccttcgtcttatggacaaagtctttaagaccatgtcccaactgaaggaggccattggctaaaatttttacatcg

SEQ ID NO: 123 - DNA, 80 bp, synthetic construct
  misc_feature 1..80: note = hANGPTL3-31 target
  source 1..80: mol_type = other DNA
gtctttttatgatctatcgctgcaaaccagtgaaatcaaagaagaagaaaaggaactgagaagaactacatataaactac

SEQ ID NO: 124 - DNA, 80 bp, synthetic construct
  misc_feature 1..80: note = hANGPTL3-32 target
  source 1..80: mol_type = other DNA
gagccaaaatcaagatttgctatgttagacgatgtaaaaattttagccaatggcctccttcagttgggacatggtcttaa

SEQ ID NO: 125 - DNA, 80 bp, synthetic construct
  misc_feature 1..80: note = hANGPTL3-33 target
  source 1..80: mol_type = other DNA
aaaaagtaatgaattaagtatgcatttctcaaactgtactttagttcttttggaaacagtgatccattccaaaaaacact

SEQ ID NO: 126 - DNA, 80 bp, synthetic construct
  misc_feature 1..80: note = hANGPTL3-34 target
  source 1..80: mol_type = other DNA
gacctagacttcttaactctatatataccaatatttgcccagaaaaggtaaggttggtaggtgaacatagttaatcatta

SEQ ID NO: 127 - DNA, 80 bp, synthetic construct
  misc_feature 1..80: note = hANGPTL3-35 target
  source 1..80: mol_type = other DNA
ggcccttcgtcttatggacaaagtctttaagaccatgtcccaactgaaggaggccattggctaaaatttttacatcgtct

SEQ ID NO: 128 - DNA, 80 bp, synthetic construct
  misc_feature 1..80: note = hANGPTL3-36 target
  source 1..80: mol_type = other DNA
atgttagacgatgtaaaaattttagccaatggcctccttcagttgggacatggtcttaaagactttgtccataagacgaa

SEQ ID NO: 129 - DNA, 80 bp, synthetic construct
  misc_feature 1..80: note = hANGPTL3-37 target
  source 1..80: mol_type = other DNA
atttgctatgttagacgatgtaaaaattttagccaatggcctccttcagttgggacatggtcttaaagactttgtccata

SEQ ID NO: 130 - DNA, 80 bp, synthetic construct
  misc_feature 1..80: note = hANGPTL3-38 target
  source 1..80: mol_type = other DNA
ttttggctctggagatagagaatcaaatgatgaattgtcttgatcaattctggaggaaataactagaggaacaataaaaa

SEQ ID NO: 131 - DNA, 80 bp, synthetic construct
  misc_feature 1..80: note = hANGPTL3-39 target
  source 1..80: mol_type = other DNA
aattgtcttgatcaattctggaggaaataactagaggaacaataaaaagaaggagcttaattgtgaacatttttatcttg

SEQ ID NO: 132 - DNA, 80 bp, synthetic construct
  misc_feature 1..80: note = hANGPTL3-40 target
  source 1..80: mol_type = other DNA
aaccttaccttttctgggcaaatattggtatatatagagttaagaagtctaggtctgcttccagaagaaaacagttccac

SEQ ID NO: 133 - DNA, 80 bp, synthetic construct
  misc_feature 1..80: note = hANGPTL3-41 target
  source 1..80: mol_type = other DNA
caaatatgttgagtttttgaaatatgtcattaatttggcccttcgtcttatggacaaagtctttaagaccatgtcccaac

SEQ ID NO: 134 - DNA, 80 bp, synthetic construct
  misc_feature 1..80: note = hANGPTL3-42 target
  source 1..80: mol_type = other DNA
aagcagacctagacttcttaactctatatataccaatatttgcccagaaaaggtaaggttggtaggtgaacatagttaat

SEQ ID NO: 135 - DNA, 80 bp, synthetic construct
  misc_feature 1..80: note = hANGPTL3-43 target
  source 1..80: mol_type = other DNA
tttgctatgttagacgatgtaaaaattttagccaatggcctccttcagttgggacatggtcttaaagactttgtccataa

SEQ ID NO: 136 - DNA, 80 bp, synthetic construct
  misc_feature 1..80: note = hANGPTL3-44 target
  source 1..80: mol_type = other DNA
ttggctaaaatttttacatcgtctaacatagcaaatcttgattttggctctggagatagagaatcaaatgatgaattgtc

SEQ ID NO: 137 - DNA, 80 bp, synthetic construct
  misc_feature 1..80: note = hANGPTL3-45 target
  source 1..80: mol_type = other DNA
taatgattaactatgttcacctaccaaccttaccttttctgggcaaatattggtatatatagagttaagaagtctaggtc

SEQ ID NO: 138 - DNA, 80 bp, synthetic construct
  misc_feature 1..80: note = hANGPTL3-46 target
  source 1..80: mol_type = other DNA
ttaacacggcttaatgattaactatgttcacctaccaaccttaccttttctgggcaaatattggtatatatagagttaag

SEQ ID NO: 139 - DNA, 80 bp, synthetic construct
  misc_feature 1..80: note = hANGPTL3-47 target
  source 1..80: mol_type = other DNA
acatttttatcttgattttcaatttcaagcaacgtggaactgttttcttctggaagcagacctagacttcttaactctat

SEQ ID NO: 140 - DNA, 80 bp, synthetic construct
  misc_feature 1..80: note = hANGPTL3-48 target
  source 1..80: mol_type = other DNA
cataaaaagactgatcaaatatgttgagtttttgaaatatgtcattaatttggcccttcgtcttatggacaaagtcttta

SEQ ID NO: 141 - DNA, 80 bp, synthetic construct
  misc_feature 1..80: note = hANGPTL3-49 target
  source 1..80: mol_type = other DNA
taacacggcttaatgattaactatgttcacctaccaaccttaccttttctgggcaaatattggtatatatagagttaaga

SEQ ID NO: 142 - DNA, 80 bp, synthetic construct
  misc_feature 1..80: note = hANGPTL3-50 target
  source 1..80: mol_type = other DNA
aggccattggctaaaatttttacatcgtctaacatagcaaatcttgattttggctctggagatagagaatcaaatgatga

SEQ ID NO: 143 - DNA, 7151 bp, synthetic construct
  misc_feature 1..7151: note = EpiRegA mRNA sequence
  source 1..7151: mol_type = other DNA
actcactatttgttttcgcgcccagttgcaaaaagtgtcgacatttgcttctgacacaactgtgttcactagcaacctcaaacagacaccgccaccatgcctgctgctaagagagtgaaactggatggatccaaccatgaccaggaatttgaccccccaaaggtttacccacctgtgccagctgagaagaggaagcccatccgcgtgctgtctctctttgatgggattgctacagggctcctggtgctgaaggacctgggcatccaagtggaccgctacattgcctccgaggtgtgtgaggactccatcacggtgggcatggtgcggcaccagggaaagatcatgtacgtcggggacgtccgcagcgtcacacagaagcatatccaggagtggggcccattcgacctggtgattggaggcagtccctgcaatgacctctccattgtcaaccctgcccgcaagggactttatgagggtactggccgcctcttctttgagttctaccgcctcctgcatgatgcgcggcccaaggagggagatgatcgccccttcttctggctctttgagaatgtggtggccatgggcgttagtgacaagagggacatctcgcgatttcttgagtctaaccccgtgatgattgacgccaaagaagtgtctgctgcacacagggcccgttacttctggggtaaccttcctggcatgaacaggcctttggcatccactgtgaatgataagctggagctgcaagagtgtctggagcacggcagaatagccaagttcagcaaagtgaggaccattaccaccaggtcaaactctataaagcagggcaaagaccagcatttccccgtgttcatgaacgagaaggaggacatcctgtggtgcactgaaatggaaagggtgtttggcttccccgtccactacacagacgtctccaacatgagccgcttggcgaggcagagactgctgggccgatcgtggagcgtgccggtcatccgccacctcttcgctccgctgaaggaatattttgcttgtgtgtctagcggcaatagtaacgctaacagccgcgggccgagcttcagcagcggcctggtgccgttaagcttgcgcggcagccatatgggccctatggagatatacaagacagtgtctgcatggaagagacagccagtgcgggtactgagcctcttcagaaacatcgacaaggtactaaagagtttgggcttcttggaaagcggttctggttctgggggaggaacgctgaagtacgtggaagatgtcacaaatgtcgtgaggagagacgtggagaaatggggcccctttgacctggtgtacggctcgacgcagcccctaggcagctcttgtgatcgctgtcccggctggtacatgttccagttccaccggatcctgcagtatgcgctgcctcgccaggagagtcagcggcccttcttctggatattcatggacaatctgctgctgactgaggatgaccaagagacaactacccgcttccttcagacagaggctgtgaccctccaggatgtccgtggcagagactaccagaatgctatgcgggtgtggagcaacattccagggctgaagagcaagcatgcgcccctgaccccaaaggaagaagagtatctgcaagcccaagtcagaagcaggagcaagctggacgccccgaaagttgacctcctggtgaagaactgccttctcccgctgagagagtacttcaagtatttttctcaaaactcacttcctcttggagggccgagctctggcgcacccccaccaagtggagggtctcctgccgggtccccaacatctactgaagaaggcaccagcgaatccgcaacgcccgagtcaggccctggtacctccacagaaccatctgaaggtagtgcgcctggttccccagctggaagccctacttccaccgaagaaggcacgtcaaccgaaccaagtgaaggatctgcccctgggaccagcactgaaccatctgagccaaaaaagaagagaaaggtaatggacaagaagtacagcatcggcctggccatcggcaccaactctgtgggctgggccgtgatcaccgacgagtacaaggtgcccagcaagaaattcaaggtgctgggcaacaccgaccggcacagcatcaagaagaacctgatcggcgccctgctgttcgacagcggagaaacagccgaggccacccggctgaagagaaccgccagaagaagatacaccagacggaagaaccggatctgctatctgcaagagatcttcagcaacgagatggccaaggtggacgacagcttcttccacagactggaagagtccttcctggtggaagaggataagaagcacgagcggcaccccatcttcggcaacatcgtggacgaggtggcctaccacgagaagtaccccaccatctaccacctgagaaagaaactggtggacagcaccgacaaggccgacctgcggctgatctatctggccctggcccacatgatcaagttccggggccacttcctgatcgagggcgacctgaaccccgacaacagcgacgtggacaagctgttcatccagctggtgcagacctacaaccagctgttcgaggaaaaccccatcaacgccagcggcgtggacgccaaggccatcctgtctgccagactgagcaagagcagacggctggaaaatctgatcgcccagctgcccggcgagaagaagaatggcctgttcggcaacctgattgccctgagcctgggcctgacccccaacttcaagagcaacttcgacctggccgaggatgccaaactgcagctgagcaaggacacctacgacgacgacctggacaacctgctggcccagatcggcgaccagtacgccgacctgtttctggccgccaagaacctgtccgacgccatcctgctgagcgacatcctgagagtgaacaccgagatcaccaaggcccccctgagcgcctctatgatcaagagatacgacgagcaccaccaggacctgaccctgctgaaagctctcgtgcggcagcagctgcctgagaagtacaaagagattttcttcgaccagagcaagaacggctacgccggctacatcgatggcggagccagccaggaagagttctacaagttcatcaagcccatcctggaaaagatggacggcaccgaggaactgctcgtgaagctgaacagagaggacctgctgcggaagcagcggaccttcgacaacggcagcatcccccaccagatccacctgggagagctgcacgccattctgcggcggcaggaagatttttacccattcctgaaggacaaccgggaaaagatcgagaagatcctgaccttccgcatcccctactacgtgggccctctggccaggggaaacagcagattcgcctggatgaccagaaagagcgaggaaaccatcaccccctggaacttcgaggaagtggtggacaagggcgccagcgcccagagcttcatcgagcggatgaccaacttcgataagaacctgcccaacgagaaggtgctgcccaagcacagcctgctgtacgagtacttcaccgtgtacaacgagctgaccaaagtgaaatacgtgaccgagggaatgagaaagcccgccttcctgagcggcgagcagaaaaaagccatcgtggacctgctgttcaagaccaaccggaaagtgaccgtgaagcagctgaaagaggactacttcaagaaaatcgagtgcttcgactccgtggaaatctccggcgtggaagatcggttcaacgcctccctgggcacataccacgatctgctgaaaattatcaaggacaaggacttcctggacaatgaggaaaacgaggacattctggaagatatcgtgctgaccctgacactgtttgaggacagagagatgatcgaggaacggctgaaaacctatgcccacctgttcgacgacaaagtgatgaagcagctgaagcggcggagatacaccggctggggcaggctgagccggaagctgatcaacggcatccgggacaagcagtccggcaagacaatcctggatttcctgaagtccgacggcttcgccaacagaaacttcatgcagctgatccacgacgacagcctgacctttaaagaggacatccagaaagcccaggtgtccggccagggcgatagcctgcacgagcacattgccaatctggccggcagccccgccattaagaagggcatcctgcagacagtgaaggtggtggacgagctcgtgaaagtgatgggccggcacaagcccgagaacatcgtgatcgaaatggccagagagaaccagaccacccagaagggacagaagaacagccgcgagagaatgaagcggatcgaagagggcatcaaagagctgggcagccagatcctgaaagaacaccccgtggaaaacacccagctgcagaacgagaagctgtacctgtactacctgcagaatgggcgggatatgtacgtggaccaggaactggacatcaaccggctgtccgactacgatgtggacgctatcgtgcctcagagctttctgaaggacgactccatcgataacaaagtgctgactcggagcgacaagaaccggggcaagagcgacaacgtgccctccgaagaggtcgtgaagaagatgaagaactactggcgccagctgctgaatgccaagctgattacccagaggaagttcgacaatctgaccaaggccgagagaggcggcctgagcgaactggataaggccggcttcatcaagagacagctggtggaaacccggcagatcacaaagcacgtggcacagatcctggactcccggatgaacactaagtacgacgagaacgacaaactgatccgggaagtgaaagtgatcaccctgaagtccaagctggtgtccgatttccggaaggatttccagttttacaaagtgcgcgagatcaacaactaccaccacgcccacgacgcctacctgaacgccgtcgtgggaaccgccctgatcaaaaagtaccctaagctggaaagcgagttcgtgtacggcgactacaaggtgtacgacgtgcggaagatgatcgccaagagcgagcaggaaatcggcaaggctaccgccaagtacttcttctacagcaacatcatgaactttttcaagaccgagattaccctggccaacggcgagatccggaagcggcctctgatcgagacaaacggcgaaacaggcgagatcgtgtgggataagggccgggactttgccaccgtgcggaaagtgctgtctatgccccaagtgaatatcgtgaaaaagaccgaggtgcagacaggcggcttcagcaaagagtctatcctgcccaagaggaacagcgacaagctgatcgccagaaagaaggactgggaccctaagaagtacggcggcttcgacagccccaccgtggcctattctgtgctggtggtggccaaagtggaaaagggcaagtccaagaaactgaagagtgtgaaagagctgctggggatcaccatcatggaaagaagcagcttcgagaagaatcccatcgactttctggaagccaagggctacaaagaagtgaaaaaggacctgatcatcaagctgcctaagtactccctgttcgagctggaaaacggccggaagagaatgctggcctctgccggcgaactgcagaagggaaacgaactggccctgccctccaaatatgtgaacttcctgtacctggccagccactatgagaagctgaagggctcccccgaggataatgagcagaaacagctgtttgtggaacagcacaaacactacctggacgagatcatcgagcagatcagcgagttctccaagagagtgatcctggccgacgctaatctggacaaggtgctgagcgcctacaacaagcacagagacaagcctatcagagagcaggccgagaatatcatccacctgtttaccctgaccaatctgggagcccctgccgccttcaagtactttgacaccaccatcgaccggaagaggtacaccagcaccaaagaggtgctggacgccaccctgatccaccagagcatcaccggcctgtacgagacacggatcgacctgtctcagctgggaggcgacgcctatccctatgacgtgcccgattatgccagcctgggcagcggctcccccaagaaaaaacgcaaggtggaagatcctaagaaaaagcggaaagtggacggcagcggcagcgagacccccggtaccagcgagagcgccacccccgagagccggacactggtgaccttcaaggatgtatttgtggacttcaccagggaggagtggaagctgctggacactgctcagcagatcgtgtacagaaatgtgatgctggagaactataagaacctggtttccttgggttatcagcttactaagccagatgtgatcctccggttggagaagggagaagagccctgagatcccaagcacgcagcaatgcagctcaaaacgcttagcctagccacacccccacgggaaacagcagtgattaacctttagcaataaacgaaagtttaactaagctatactaaccccagggttggtcaatttcgtgccagccacaccctggtactgcatgcacgcaatgctagctgcccctttcccgtcctgggcaccccgagtctcccccgaccccgggtcccaggtatgctcccacctccacctgccccactcaccacctctgctagttccagacacctccgagacgaggaaaaaaaaaaaaaaaaaaaaaaaaaaaaaaaaaaaaaaaaaaaaaaaaaaaaaaaaaaaaaaaaaaaaaaaaaaaaaaaaaaaaaaaaaaaaaaaaaaaaaaaaaaaaaaaaaaaaaaaaaaaaaaaaaaaaaaaaaaaaaaaaaaaaaaaaaaaaaaaaaaaaaaaaaaaaaaaaaaaaaaaaaaaaaaaaaaaaaaaaaaaaaaaaaaaaaaaaaaaaaaaaaaaaaaaaaaaaaaaaaaaaaaaaaaaaaaaaaaaaaaaaaaaaaaaaaaaaaaaaaaaaaaaaaaaaaaaaaaaaaaaaaaaaaaaaaaaaaaaaaaaaaaaaaaaaaaaaaaaaaaaaaaaaaaaaaaaaaaaaaaaaaaaaaaaaaaaaaaaaaaaaaaaaaaaaaa

SEQ ID NO: 144 - protein, 2123 aa, synthetic construct
  REGION 1..2123: note = EpiRegA AA sequence
  SITE 2123: note = misc_feature - Xaa =
MPAAKRVKLDGSNHDQEFDPPKVYPPVPAEKRKPIRVLSLFDGIATGLLVLKDLGIQVDRYIASEVCEDSITVGMVRHQGKIMYVGDVRSVTQKHIQEWGPFDLVIGGSPCNDLSIVNPARKGLYEGTGRLFFEFYRLLHDARPKEGDDRPFFWLFENVVAMGVSDKRDISRFLESNPVMIDAKEVSAAHRARYFWGNLPGMNRPLASTVNDKLELQECLEHGRIAKFSKVRTITTRSNSIKQGKDQHFPVFMNEKEDILWCTEMERVFGFPVHYTDVSNMSRLARQRLLGRSWSVPVIRHLFAPLKEYFACVSSGNSNANSRGPSFSSGLVPLSLRGSHMGPMEIYKTVSAWKRQPVRVLSLFRNIDKVLKSLGFLESGSGSGGGTLKYVEDVTNVVRRDVEKWGPFDLVYGSTQPLGSSCDRCPGWYMFQFHRILQYALPRQESQRPFFWIFMDNLLLTEDDQETTTRFLQTEAVTLQDVRGRDYQNAMRVWSNIPGLKSKHAPLTPKEEEYLQAQVRSRSKLDAPKVDLLVKNCLLPLREYFKYFSQNSLPLGGPSSGAPPPSGGSPAGSPTSTEEGTSESATPESGPGTSTEPSEGSAPGSPAGSPTSTEEGTSTEPSEGSAPGTSTEPSEPKKKRKVMDKKYSIGLAIGTNSVGWAVITDEYKVPSKKFKVLGNTDRHSIKKNLIGALLFDSGETAEATRLKRTARRRYTRRKNRICYLQEIFSNEMAKVDDSFFHRLEESFLVEEDKKHERHPIFGNIVDEVAYHEKYPTIYHLRKKLVDSTDKADLRLIYLALAHMIKFRGHFLIEGDLNPDNSDVDKLFIQLVQTYNQLFEENPINASGVDAKAILSARLSKSRRLENLIAQLPGEKKNGLFGNLIALSLGLTPNFKSNFDLAEDAKLQLSKDTYDDDLDNLLAQIGDQYADLFLAAKNLSDAILLSDILRVNTEITKAPLSASMIKRYDEHHQDLTLLKALVRQQLPEKYKEIFFDQSKNGYAGYIDGGASQEEFYKFIKPILEKMDGTEELLVKLNREDLLRKQRTFDNGSIPHQIHLGELHAILRRQEDFYPFLKDNREKIEKILTFRIPYYVGPLARGNSRFAWMTRKSEETITPWNFEEVVDKGASAQSFIERMTNFDKNLPNEKVLPKHSLLYEYFTVYNELTKVKYVTEGMRKPAFLSGEQKKAIVDLLFKTNRKVTVKQLKEDYFKKIECFDSVEISGVEDRFNASLGTYHDLLKIIKDKDFLDNEENEDILEDIVLTLTLFEDREMIEERLKTYAHLFDDKVMKQLKRRRYTGWGRLSRKLINGIRDKQSGKTILDFLKSDGFANRNFMQLIHDDSLTFKEDIQKAQVSGQGDSLHEHIANLAGSPAIKKGILQTVKVVDELVKVMGRHKPENIVIEMARENQTTQKGQKNSRERMKRIEEGIKELGSQILKEHPVENTQLQNEKLYLYYLQNGRDMYVDQELDINRLSDYDVDAIVPQSFLKDDSIDNKVLTRSDKNRGKSDNVPSEEVVKKMKNYWRQLLNAKLITQRKFDNLTKAERGGLSELDKAGFIKRQLVETRQITKHVAQILDSRMNTKYDENDKLIREVKVITLKSKLVSDFRKDFQFYKVREINNYHHAHDAYLNAVVGTALIKKYPKLESEFVYGDYKVYDVRKMIAKSEQEIGKATAKYFFYSNIMNFFKTEITLANGEIRKRPLIETNGETGEIVWDKGRDFATVRKVLSMPQVNIVKKTEVQTGGFSKESILPKRNSDKLIARKKDWDPKKYGGFDSPTVAYSVLVVAKVEKGKSKKLKSVKELLGITIMERSSFEKNPIDFLEAKGYKEVKKDLIIKLPKYSLFELENGRKRMLASAGELQKGNELALPSKYVNFLYLASHYEKLKGSPEDNEQKQLFVEQHKHYLDEIIEQISEFSKRVILADANLDKVLSAYNKHRDKPIREQAENIIHLFTLTNLGAPAAFKYFDTTIDRKRYTSTKEVLDATLIHQSITGLYETRIDLSQLGGDAYPYDVPDYASLGSGSPKKKRKVEDPKKKRKVDGSGSETPGTSESATPESRTLVTFKDVFVDFTREEWKLLDTAQQIVYRNVMLENYKNLVSLGYQLTKPDVILRLEKGEEPX

SEQ ID NO: 145 - DNA, 7540 bp, synthetic construct
  misc_feature 1..7540: note = EpiRegB mRNA sequence
  source 1..7540: mol_type = other DNA
actcactatttgttttcgcgcccagttgcaaaaagtgtcgacatttgcttctgacacaactgtgttcactagcaacctcaaacagacaccttaattaagccaccatgccaaaaaagaagagaaaggtaatggacaagaagtacagcatcggcctggccatcggcaccaactctgtgggctgggccgtgatcaccgacgagtacaaggtgcccagcaagaaattcaaggtgctgggcaacaccgaccggcacagcatcaagaagaacctgatcggcgccctgctgttcgacagcggagaaacagccgaggccacccggctgaagagaaccgccagaagaagatacaccagacggaagaaccggatctgctatctgcaagagatcttcagcaacgagatggccaaggtggacgacagcttcttccacagactggaagagtccttcctggtggaagaggataagaagcacgagcggcaccccatcttcggcaacatcgtggacgaggtggcctaccacgagaagtaccccaccatctaccacctgagaaagaaactggtggacagcaccgacaaggccgacctgcggctgatctatctggccctggcccacatgatcaagttccggggccacttcctgatcgagggcgacctgaaccccgacaacagcgacgtggacaagctgttcatccagctggtgcagacctacaaccagctgttcgaggaaaaccccatcaacgccagcggcgtggacgccaaggccatcctgtctgccagactgagcaagagcagacggctggaaaatctgatcgcccagctgcccggcgagaagaagaatggcctgttcggcaacctgattgccctgagcctgggcctgacccccaacttcaagagcaacttcgacctggccgaggatgccaaactgcagctgagcaaggacacctacgacgacgacctggacaacctgctggcccagatcggcgaccagtacgccgacctgtttctggccgccaagaacctgtccgacgccatcctgctgagcgacatcctgagagtgaacaccgagatcaccaaggcccccctgagcgcctctatgatcaagagatacgacgagcaccaccaggacctgaccctgctgaaagctctcgtgcggcagcagctgcctgagaagtacaaagagattttcttcgaccagagcaagaacggctacgccggctacatcgatggcggagccagccaggaagagttctacaagttcatcaagcccatcctggaaaagatggacggcaccgaggaactgctcgtgaagctgaacagagaggacctgctgcggaagcagcggaccttcgacaacggcagcatcccccaccagatccacctgggagagctgcacgccattctgcggcggcaggaagatttttacccattcctgaaggacaaccgggaaaagatcgagaagatcctgaccttccgcatcccctactacgtgggccctctggccaggggaaacagcagattcgcctggatgaccagaaagagcgaggaaaccatcaccccctggaacttcgaggaagtggtggacaagggcgccagcgcccagagcttcatcgagcggatgaccaacttcgataagaacctgcccaacgagaaggtgctgcccaagcacagcctgctgtacgagtacttcaccgtgtacaacgagctgaccaaagtgaaatacgtgaccgagggaatgagaaagcccgccttcctgagcggcgagcagaaaaaagccatcgtggacctgctgttcaagaccaaccggaaagtgaccgtgaagcagctgaaagaggactacttcaagaaaatcgagtgcttcgactccgtggaaatctccggcgtggaagatcggttcaacgcctccctgggcacataccacgatctgctgaaaattatcaaggacaaggacttcctggacaatgaggaaaacgaggacattctggaagatatcgtgctgaccctgacactgtttgaggacagagagatgatcgaggaacggctgaaaacctatgcccacctgttcgacgacaaagtgatgaagcagctgaagcggcggagatacaccggctggggcaggctgagccggaagctgatcaacggcatccgggacaagcagtccggcaagacaatcctggatttcctgaagtccgacggcttcgccaacagaaacttcatgcagctgatccacgacgacagcctgacctttaaagaggacatccagaaagcccaggtgtccggccagggcgatagcctgcacgagcacattgccaatctggccggcagccccgccattaagaagggcatcctgcagacagtgaaggtggtggacgagctcgtgaaagtgatgggccggcacaagcccgagaacatcgtgatcgaaatggccagagagaaccagaccacccagaagggacagaagaacagccgcgagagaatgaagcggatcgaagagggcatcaaagagctgggcagccagatcctgaaagaacaccccgtggaaaacacccagctgcagaacgagaagctgtacctgtactacctgcagaatgggcgggatatgtacgtggaccaggaactggacatcaaccggctgtccgactacgatgtggacgctatcgtgcctcagagctttctgaaggacgactccatcgataacaaagtgctgactcggagcgacaagaaccggggcaagagcgacaacgtgccctccgaagaggtcgtgaagaagatgaagaactactggcgccagctgctgaatgccaagctgattacccagaggaagttcgacaatctgaccaaggccgagagaggcggcctgagcgaactggataaggccggcttcatcaagagacagctggtggaaacccggcagatcacaaagcacgtggcacagatcctggactcccggatgaacactaagtacgacgagaacgacaaactgatccgggaagtgaaagtgatcaccctgaagtccaagctggtgtccgatttccggaaggatttccagttttacaaagtgcgcgagatcaacaactaccaccacgcccacgacgcctacctgaacgccgtcgtgggaaccgccctgatcaaaaagtaccctaagctggaaagcgagttcgtgtacggcgactacaaggtgtacgacgtgcggaagatgatcgccaagagcgagcaggaaatcggcaaggctaccgccaagtacttcttctacagcaacatcatgaactttttcaagaccgagattaccctggccaacggcgagatccggaagcggcctctgatcgagacaaacggcgaaacaggcgagatcgtgtgggataagggccgggactttgccaccgtgcggaaagtgctgtctatgccccaagtgaatatcgtgaaaaagaccgaggtgcagacaggcggcttcagcaaagagtctatcctgcccaagaggaacagcgacaagctgatcgccagaaagaaggactgggaccctaagaagtacggcggcttcgacagccccaccgtggcctattctgtgctggtggtggccaaagtggaaaagggcaagtccaagaaactgaagagtgtgaaagagctgctggggatcaccatcatggaaagaagcagcttcgagaagaatcccatcgactttctggaagccaagggctacaaagaagtgaaaaaggacctgatcatcaagctgcctaagtactccctgttcgagctggaaaacggccggaagagaatgctggcctctgccggcgaactgcagaagggaaacgaactggccctgccctccaaatatgtgaacttcctgtacctggccagccactatgagaagctgaagggctcccccgaggataatgagcagaaacagctgtttgtggaacagcacaaacactacctggacgagatcatcgagcagatcagcgagttctccaagagagtgatcctggccgacgctaatctggacaaggtgctgagcgcctacaacaagcacagagacaagcctatcagagagcaggccgagaatatcatccacctgtttaccctgaccaatctgggagcccctgccgccttcaagtactttgacaccaccatcgaccggaagaggtacaccagcaccaaagaggtgctggacgccaccctgatccaccagagcatcaccggcctgtacgagacacggatcgacctgtctcagctgggaggcgacgcctatccctatgacgtgcccgattatgccagcctgggcagcggctcccccaagaaaaaacgcaaggtggaagatcctaagaaaaagcggaaagtggacggcggagggccgagctctggcgcacccccaccaagtggagggtctcctgccgggtccccaacatctactgaagaaggcaccagcgaatccgcaacgcccgagtcaggccctggtacctccacagaaccatctgaaggtagtgcgcctggttccccagctggaagccctacttccaccgaagaaggcacgtcaaccgaaccaagtgaaggatctgcccctgggaccagcactgaaccatctgagatgaacaattcccagggaagagtgaccttcgaggacgtgaccgtgaacttcacccaaggcgagtggcagagactgaaccccgagcagagaaacctgtaccgggacgtgatgctggaaaactacagcaacctggtgtccgtcggccagggcgagacaacaaagcctgacgtgatcctgcggctggaacagggcaaagagccttggctggaagaggaagaggtgctcggatctggcagagccgagaagaatggcgatatcggcggacagatctggaagccaaaggatgtgaaagagagtctcagcggcagcgagacccccggtaccagcgagggcggccctagcagcggcgcccctccccctagcggcggcagccctgccggatcccctacaagcaccgaagaaggcacaagcgagtccgctacccctgagtccggccctggcacctccacagagcctagcgagggatccgctcctggatcccctgccggaagccctacctccaccgaggagggcacaagcaccgagccttccgagggcagcgcccccggaacaagcaccgaacctagcgagagcgccacccccgagagcatgttcgaaaccgtgcctgtgtggaggagacagccagtccgggtgctgtccctttttgaagacatcaagaaagagctgacgagtttgggctttttggaaagtggttctgacccgggacaactgaagcatgtggttgatgtcacagacacagtgaggaaggatgtggaggagtggggacccttcgatcttgtgtacggcgccacacctcccctgggccacacctgtgaccgtcctcccagctggtacctgttccagttccaccggctcctgcagtacgcacggcccaagccaggcagccccaggcccttcttctggatgttcgtggacaatctggtgctgaacaaggaagacctggacgtcgcatctcgcttcctggagatggagccagtcaccatcccagatgtccacggcggatccttgcagaatgctgtccgcgtgtggagcaacatcccagccataaggagcagcaggcactgggctctggtttcggaagaagaattgtccctgctggcccagaacaagcagagctcgaagctcgcggccaagtggcccaccaagctggtgaagaactgctttctccccctaagagaatatttcaagtatttttcaacagaactcacttcctctttatctagcggcaatagtaacgctaacagccgcgggccgagcttcagcagcggcctggtgccgttaagcttgcgcggcagccatatgaaccatgaccaggaatttgaccccccaaaggtttacccacctgtgccagctgagaagaggaagcccatccgcgtgctgtctctctttgatgggattgctacagggctcctggtgctgaaggacctgggcatccaagtggaccgctacattgcctccgaggtgtgtgaggactccatcacggtgggcatggtgcggcaccagggaaagatcatgtacgtcggggacgtccgcagcgtcacacagaagcatatccaggagtggggcccattcgacctggtgattggaggcagtccctgcaatgacctctccattgtcaaccctgcccgcaagggactttatgagggtactggccgcctcttctttgagttctaccgcctcctgcatgatgcgcggcccaaggagggagatgatcgccccttcttctggctctttgagaatgtggtggccatgggcgttagtgacaagagggacatctcgcgatttcttgagtctaaccccgtgatgattgacgccaaagaagtgtctgctgcacacagggcccgttacttctggggtaaccttcctggcatgaacaggcctttggcatccactgtgaatgataagctggagctgcaagagtgtctggagcacggcagaatagccaagttcagcaaagtgaggaccattaccaccaggtcaaactctataaagcagggcaaagaccagcatttccccgtcttcatgaacgagaaggaggacatcctgtggtgcactgaaatggaaagggtgtttggcttccccgtccactacacagacgtctccaacatgagccgcttggcgaggcagagactgctgggccgatcgtggagcgtgccggtcatccgccacctcttcgctccgctgaaggaatattttgcttgtgtgctcgaggctactaacttcagcctgctgaagcaggctggagacgtggaggagaaccctggacctatgcattaatgagatcccaagcacgcagcaatgcagctcaaaacgcttagcctagccacacccccacgggaaacagcagtgattaacctttagcaataaacgaaagtttaactaagctatactaaccccagggttggtcaatttcgtgccagccacaccctggtactgcatgcacgcaatgctagctgcccctttcccgtcctgggcaccccgagtctcccccgaccccgggtcccaggtatgctcccacctccacctgccccactcaccacctctgctagttccagacacctccgagacgaggaaaaaaaaaaaaaaaaaaaaaaaaaaaaaaaaaaaaaaaaaaaaaaaaaaaaaaaaaaaaaaaaaaaaaaaaaaaaaaaaaaaaaaaaaaaaaaaaaaaaaaaaaaaaaaaaaaaaaaaaaaaaaaaaaaaaaaaaaaaaaaaaaaaaaaaaaaaaaaaaaaaaaaaaaaaaaaaaaaaaaaaaaaaaaaaaaaaaaaaaaaaaaaaaaaaaaaaaaaaaaaaaaaaaaaaaaaaaaaaaaaaaaaaaaaaaaaaaaaaaaaaaaaaaaaaaaaaaaaaaaaaaaaaaaaaaaaaaaaaaaaaaaaaaaaaaaaaaaaaaaaaaaaaaaaaaaaaaaaaaaaaaaaaaaaaaaaaaaaaaaaaaaaaaaaaaaaaaaaaaaaaaaaaaaaaaaa

SEQ ID NO: 146 - protein, 2249 aa, synthetic construct
  REGION 1..2249: note = EpiRegB AA sequence
  SITE 2249: note = misc_feature - Xaa =
MPKKKRKVMDKKYSIGLAIGTNSVGWAVITDEYKVPSKKFKVLGNTDRHSIKKNLIGALLFDSGETAEATRLKRTARRRYTRRKNRICYLQEIFSNEMAKVDDSFFHRLEESFLVEEDKKHERHPIFGNIVDEVAYHEKYPTIYHLRKKLVDSTDKADLRLIYLALAHMIKFRGHFLIEGDLNPDNSDVDKLFIQLVQTYNQLFEENPINASGVDAKAILSARLSKSRRLENLIAQLPGEKKNGLFGNLIALSLGLTPNFKSNFDLAEDAKLQLSKDTYDDDLDNLLAQIGDQYADLFLAAKNLSDAILLSDILRVNTEITKAPLSASMIKRYDEHHQDLTLLKALVRQQLPEKYKEIFFDQSKNGYAGYIDGGASQEEFYKFIKPILEKMDGTEELLVKLNREDLLRKQRTFDNGSIPHQIHLGELHAILRRQEDFYPFLKDNREKIEKILTFRIPYYVGPLARGNSRFAWMTRKSEETITPWNFEEVVDKGASAQSFIERMTNFDKNLPNEKVLPKHSLLYEYFTVYNELTKVKYVTEGMRKPAFLSGEQKKAIVDLLFKTNRKVTVKQLKEDYFKKIECFDSVEISGVEDRFNASLGTYHDLLKIIKDKDFLDNEENEDILEDIVLTLTLFEDREMIEERLKTYAHLFDDKVMKQLKRRRYTGWGRLSRKLINGIRDKQSGKTILDFLKSDGFANRNFMQLIHDDSLTFKEDIQKAQVSGQGDSLHEHIANLAGSPAIKKGILQTVKVVDELVKVMGRHKPENIVIEMARENQTTQKGQKNSRERMKRIEEGIKELGSQILKEHPVENTQLQNEKLYLYYLQNGRDMYVDQELDINRLSDYDVDAIVPQSFLKDDSIDNKVLTRSDKNRGKSDNVPSEEVVKKMKNYWRQLLNAKLITQRKFDNLTKAERGGLSELDKAGFIKRQLVETRQITKHVAQILDSRMNTKYDENDKLIREVKVITLKSKLVSDFRKDFQFYKVREINNYHHAHDAYLNAVVGTALIKKYPKLESEFVYGDYKVYDVRKMIAKSEQEIGKATAKYFFYSNIMNFFKTEITLANGEIRKRPLIETNGETGEIVWDKGRDFATVRKVLSMPQVNIVKKTEVQTGGFSKESILPKRNSDKLIARKKDWDPKKYGGFDSPTVAYSVLVVAKVEKGKSKKLKSVKELLGITIMERSSFEKNPIDFLEAKGYKEVKKDLIIKLPKYSLFELENGRKRMLASAGELQKGNELALPSKYVNFLYLASHYEKLKGSPEDNEQKQLFVEQHKHYLDEIIEQISEFSKRVILADANLDKVLSAYNKHRDKPIREQAENIIHLFTLTNLGAPAAFKYFDTTIDRKRYTSTKEVLDATLIHQSITGLYETRIDLSQLGGDAYPYDVPDYASLGSGSPKKKRKVEDPKKKRKVDGGGPSSGAPPPSGGSPAGSPTSTEEGTSESATPESGPGTSTEPSEGSAPGSPAGSPTSTEEGTSTEPSEGSAPGTSTEPSEMNNSQGRVTFEDVTVNFTQGEWQRLNPEQRNLYRDVMLENYSNLVSVGQGETTKPDVILRLEQGKEPWLEEEEVLGSGRAEKNGDIGGQIWKPKDVKESLSGSETPGTSEGGPSSGAPPPSGGSPAGSPTSTEEGTSESATPESGPGTSTEPSEGSAPGSPAGSPTSTEEGTSTEPSEGSAPGTSTEPSESATPESMFETVPVWRRQPVRVLSLFEDIKKELTSLGFLESGSDPGQLKHVVDVTDTVRKDVEEWGPFDLVYGATPPLGHTCDRPPSWYLFQFHRLLQYARPKPGSPRPFFWMFVDNLVLNKEDLDVASRFLEMEPVTIPDVHGGSLQNAVRVWSNIPAIRSSRHWALVSEEELSLLAQNKQSSKLAAKWPTKLVKNCFLPLREYFKYFSTELTSSLSSGNSNANSRGPSFSSGLVPLSLRGSHMNHDQEFDPPKVYPPVPAEKRKPIRVLSLFDGIATGLLVLKDLGIQVDRYIASEVCEDSITVGMVRHQGKIMYVGDVRSVTQKHIQEWGPFDLVIGGSPCNDLSIVNPARKGLYEGTGRLFFEFYRLLHDARPKEGDDRPFFWLFENVVAMGVSDKRDISRFLESNPVMIDAKEVSAAHRARYFWGNLPGMNRPLASTVNDKLELQECLEHGRIAKFSKVRTITTRSNSIKQGKDQHFPVFMNEKEDILWCTEMERVFGFPVHYTDVSNMSRLARQRLLGRSWSVPVIRHLFAPLKEYFACVLEATNFSLLKQAGDVEENPGPMHX